European Patent Specification EP 4 075 971 B1, published January 28, 2026. Title: METHOD FOR INCREASING LONGEVITY AND/OR BUD OPENING OF CUT FLOWERS. Applicant: Letavis AB. The sequence listing filed with the application follows.

SEQUENCE LISTING (24 sequences)

SEQ ID NO: 1 - protein, 9 aa, Homo sapiens
  MOD_RES (9)..(9): AMIDATION
CYIQNCPLG

SEQ ID NO: 2 - protein, 10 aa, Artificial sequence
  Oxytocin fragments and variants
  MISC_FEATURE (1)..(1): X1 can be Cys or nothing
  MISC_FEATURE (2)..(2): X2 can be Tyr, Phe or nothing
  MISC_FEATURE (3)..(3): X3 can be Ile, Val, Hoph, Phe, Cha or nothing
  MISC_FEATURE (4)..(4): X4 can be Gln, Ser, Thr, Cit, Arg or Daba
  MISC_FEATURE (7)..(7): X5 (position 7) can be Pro or nothing
  MISC_FEATURE (8)..(8): X6 (position 8) can be Ile, Leu, nothing, Val, Hos, Daba, Thr, Arg or Cit
  MISC_FEATURE (9)..(9): X7 (position 9) can be Gly, nothing or Ala
  MOD_RES (10)..(10): AMIDATION
  MISC_FEATURE (10)..(10): X8 (position 10) can be Gly or nothing
XXXXNCXXXX

SEQ ID NO: 3 - protein, 9 aa, Bird
  MOD_RES (9)..(9): AMIDATION
CYIQNCPIG

SEQ ID NO: 4 - protein, 9 aa, Fish
  MOD_RES (9)..(9): AMIDATION
CYISNCPIG

SEQ ID NO: 5 - protein, 9 aa, Eisenia foetida
  MOD_RES (9)..(9): AMIDATION
CFVRNCPTG

SEQ ID NO: 6 - protein, 9 aa, non mammalian vertebrates, fetal mammals
  MOD_RES (9)..(9): AMIDATION
CYIQNCPRG

SEQ ID NO: 7 - protein, 9 aa, Homo sapiens
  MOD_RES (9)..(9): AMIDATION
CYFQNCPRG

SEQ ID NO: 8 - protein, 6 aa, Artificial sequence
  Oxytocin fragment
  MOD_RES (6)..(6): AMIDATION
CYIQNC

SEQ ID NO: 9 - protein, 7 aa, Artificial sequence
  oxytocin fragment
  MOD_RES (7)..(7): AMIDATION
CYIQNCP

SEQ ID NO: 10 - protein, 8 aa, Artificial sequence
  Oxytocin fragment
  MOD_RES (8)..(8): AMIDATION
CYIQNCPL

SEQ ID NO: 11 - protein, 8 aa, Artificial sequence
  Oxytocin fragment
  MOD_RES (8)..(8): AMIDATION
YIQNCPLG

SEQ ID NO: 12 - protein, 7 aa, Artificial sequence
  Oxytocin fragment
  MOD_RES (7)..(7): AMIDATION
IQNCPLG

SEQ ID NO: 13 - protein, 6 aa, Artificial sequence
  Oxytocin fragment
  MOD_RES (6)..(6): AMIDATION
QNCPLG

SEQ ID NO: 14 - protein, 5 aa, Artificial sequence
  Oxytocin fragment
  MOD_RES (5)..(5): AMIDATION
IQNCP

SEQ ID NO: 15 - protein, 10 aa, Artificial sequence
  Oxytocin variant
  MOD_RES (10)..(10): AMIDATION
CYIQNCPLGG

SEQ ID NO: 16 - protein, 6 aa, Artificial sequence
  Oxytocin variant
  MOD_RES (6)..(6): AMIDATION
QNCPLL

SEQ ID NO: 17 - protein, 9 aa, Artificial sequence
  Oxytocin variant
  MOD_RES (9)..(9): AMIDATION
CYVTNCPLG

SEQ ID NO: 18 - protein, 9 aa, Artificial sequence
  Oxytocin variant
  MISC_FEATURE (3)..(3): X is Hoph
  MOD_RES (9)..(9): AMIDATION
CYXTNCPVG

SEQ ID NO: 19 - protein, 9 aa, Artificial sequence
  Oxytocin variant
  MISC_FEATURE (4)..(4): X is Cit
  MOD_RES (9)..(9): AMIDATION
CYFXNCPLG

SEQ ID NO: 20 - protein, 9 aa, Artificial sequence
  Oxytocin variant
  MISC_FEATURE (3)..(3): X is Cha
  MISC_FEATURE (8)..(8): X is Hos
  MOD_RES (9)..(9): AMIDATION
CYXRNCPXA

SEQ ID NO: 21 - protein, 9 aa, Artificial sequence
  Oxytocin variant
  MISC_FEATURE (4)..(4): X is Daba
  MISC_FEATURE (8)..(8): X is Daba
  MOD_RES (9)..(9): AMIDATION
CYVXNCPXA

SEQ ID NO: 22 - protein, 9 aa, Artificial sequence
  Oxytocin variant
  MISC_FEATURE (3)..(3): X is Hoph
  MISC_FEATURE (4)..(4): X is Daba
  MISC_FEATURE (8)..(8): X is Cit
  MOD_RES (9)..(9): AMIDATION
CYXXNCPXA

SEQ ID NO: 23 - protein, 9 aa, Artificial sequence
  Oxytocin variant
  MOD_RES (9)..(9): AMIDATION
CYFRNCPVA

SEQ ID NO: 24 - protein, 9 aa, Artificial sequence
  Oxytocin variant
  MISC_FEATURE (3)..(3): X is Cha
  MISC_FEATURE (4)..(4): X is Cit
  MOD_RES (9)..(9): AMIDATION
CYXXNCPRG